European Patent Application EP 4 733 397 A2, published April 29, 2026. Title: COMPOSITIONS AND METHODS FOR INTERNALIZING ENZYMES. Applicant: Regeneron Pharmaceuticals, Inc. The sequence listing filed with the application follows.

SEQUENCE LISTING (81 sequences)

SEQ ID NO: 1 - protein, 952 aa, Homo sapiens
MGVRHPPCSHRLLAVCALVSLATAALLGHILLHDFLLVPRELSGSSPVLEETHPAHQQGASRPGPRDAQAHPGRPRAVPTQCDVPPNSRFDCAPDKAITQEQCEARGCCYIPAKQGLQGAQMGQPWCFFPPSYPSYKLENLSSSEMGYTATLTRTTPTFFPKDILTLRLDVMMETENRLHFTIKDPANRRYEVPLETPHVHSRAPSPLYSVEFSEEPFGVIVRRQLDGRVLLNTTVAPLFFADQFLQLSTSLPSQYITGLAEHLSPLMLSTSWTRITLWNRDLAPTPGANLYGSHPFYLALEDGGSAHGVFLLNSNAMDVVLQPSPALSWRSTGGILDVYIFLGPEPKSVVQQYLDVVGYPFMPPYWGLGFHLCRWGYSSTAITRQVVENMTRAHFPLDVQWNDLDYMDSRRDFTFNKDGFRDFPAMVQELHQGGRRYMMIVDPAISSSGPAGSYRPYDEGLRRGVFITNETGQPLIGKVWPGSTAFPDFTNPTALAWWEDMVAEFHDQVPFDGMWIDMNEPSNFIRGSEDGCPNNELENPPYVPGVVGGTLQAATICASSHQFLSTHYNLHNLYGLTEAIASHRALVKARGTRPFVISRSTFAGHGRYAGHWTGDVWSSWEQLASSVPEILQFNLLGVPLVGADVCGFLGNTSEELCVRWTQLGAFYPFMRNHNSLLSLPQEPYSFSEPAQQAMRKALTLRYALLPHLYTLFHQAHVAGETVARPLFLEFPKDSSTWTVDHQLLWGEALLITPVLQAGKAEVTGYFPLGTWYDLQTVPVEALGSLPPPPAAPREPAIHSEGQWVTLPAPLDTINVHLRAGYIIPLQGPGLTTTESRQQPMALAVALTKGGEARGELFWDDGESLEVLERGAYTQVIFLARNNTIVNELVRVTSEGAGLQLQKVTVLGVATAPQQVLSNGVPVSNFTYSPDTKVLDICVSLLMGEQFLVSWC

SEQ ID NO: 2 - protein, 245 aa, synthetic construct
EVKLVESGGGLVQPGGSLKLSCATSGFTFSDYYMSWVRQTPEKRLEWVAYISSSGGSTYYSDTVKGQFTISRDNAKNTLYLQMSRLKSEDTAMYYCARREDYDGRLTYWGQGTLVTISAGGSGGGGSGGGGSGGDIVLTQSPASLAVSLGQRATISCRASKSVSTSGYSYMNWYQQKPGQPPKVLIYLASKLESGVPARFSGSGSGTDFTLNIHPVEEEDAATYYCQHSRELPYTFGGGTKLEIK

SEQ ID NO: 3 - DNA, 21 bp, synthetic construct
  source 1..21: mol_type = other DNA
ggaacccctagtgatggagtt

SEQ ID NO: 4 - DNA, 16 bp, synthetic construct
  source 1..16: mol_type = other DNA
cggcctcagtgagcga

SEQ ID NO: 5 - DNA, 21 bp, synthetic construct
  source 1..21: mol_type = other DNA
cactccctctctgcgcgctcg

SEQ ID NO: 6 - DNA, 141 bp, synthetic construct
  source 1..141: mol_type = other DNA
cctgcaggcagctgcgcgctcgctcgctcactgaggccgcccgggcaaagcccgggcgtcgggcgacctttggtcgcccggcctcagtgagcgagcgagcgcgcagagagggagtggccaactccatcactaggggttcct

SEQ ID NO: 7 - DNA, 141 bp, synthetic construct
  source 1..141: mol_type = other DNA
aggaacccctagtgatggagttggccactccctctctgcgcgctcgctcgctcactgaggccgggcgaccaaaggtcgcccgacgcccgggctttgcccgggcggcctcagtgagcgagcgagcgcgcagctgcctgcagg

SEQ ID NO: 8 - DNA, 224 bp, synthetic construct
  source 1..224: mol_type = other DNA
gtctgtctgcacatttcgtagagcgagtgttccgatactctaatctccctaggcaaggttcatatttgtgtaggttacttattctccttttgttgactaagtcaataatcagaatcagcaggtttggagtcagcttggcagggatcagcagcctgggttggaaggagggggtataaaagccccttcaccaggagaagccgtcacacagatccacaagctcctga

SEQ ID NO: 9 - DNA, 72 bp, synthetic construct
  source 1..72: mol_type = other DNA
gggggaggctgctggtgaatattaaccaaggtcaccccagttatcggaggagcaaacaggggctaagtccac

SEQ ID NO: 10 - protein, 1133 aa, synthetic construct
EVKLVESGGGLVQPGGSLKLSCATSGFTFSDYYMSWVRQTPEKRLEWVAYISSSGGSTYYSDTVKGQFTISRDNAKNTLYLQMSRLKSEDTAMYYCARREDYDGRLTYWGQGTLVTISAGGSGGGGSGGGGSGGDIVLTQSPASLAVSLGQRATISCRASKSVSTSGYSYMNWYQQKPGQPPKVLIYLASKLESGVPARFSGSGSGTDFTLNIHPVEEEDAATYYCQHSRELPYTFGGGTKLEIKGGGGSAHPGRPRAVPTQCDVPPNSRFDCAPDKAITQEQCEARGCCYIPAKQGLQGAQMGQPWCFFPPSYPSYKLENLSSSEMGYTATLTRTTPTFFPKDILTLRLDVMMETENRLHFTIKDPANRRYEVPLETPHVHSRAPSPLYSVEFSEEPFGVIVRRQLDGRVLLNTTVAPLFFADQFLQLSTSLPSQYITGLAEHLSPLMLSTSWTRITLWNRDLAPTPGANLYGSHPFYLALEDGGSAHGVFLLNSNAMDVVLQPSPALSWRSTGGILDVYIFLGPEPKSVVQQYLDVVGYPFMPPYWGLGFHLCRWGYSSTAITRQVVENMTRAHFPLDVQWNDLDYMDSRRDFTFNKDGFRDFPAMVQELHQGGRRYMMIVDPAISSSGPAGSYRPYDEGLRRGVFITNETGQPLIGKVWPGSTAFPDFTNPTALAWWEDMVAEFHDQVPFDGMWIDMNEPSNFIRGSEDGCPNNELENPPYVPGVVGGTLQAATICASSHQFLSTHYNLHNLYGLTEAIASHRALVKARGTRPFVISRSTFAGHGRYAGHWTGDVWSSWEQLASSVPEILQFNLLGVPLVGADVCGFLGNTSEELCVRWTQLGAFYPFMRNHNSLLSLPQEPYSFSEPAQQAMRKALTLRYALLPHLYTLFHQAHVAGETVARPLFLEFPKDSSTWTVDHQLLWGEALLITPVLQAGKAEVTGYFPLGTWYDLQTVPVEALGSLPPPPAAPREPAIHSEGQWVTLPAPLDTINVHLRAGYIIPLQGPGLTTTESRQQPMALAVALTKGGEARGELFWDDGESLEVLERGAYTQVIFLARNNTIVNELVRVTSEGAGLQLQKVTVLGVATAPQQVLSNGVPVSNFTYSPDTKVLDICVSLLMGEQFLVSWC

SEQ ID NO: 11 - DNA, 3489 bp, synthetic construct
  source 1..3489: mol_type = other DNA
atgcacagacctagacgtcgtggaactcgtccacctccactggcactgctcgctgctctcctcctggctgcacgtggtgctgatgcagaagtgaagctggtggagtctgggggaggcttagtgcagcctggagggtccctgaaactctcctgtgcaacctctggattcactttcagtgactattacatgtcttgggttcgccagactccagagaagaggctggagtgggtcgcatatattagtagtagtggtggtagcacctattattcagacactgtaaagggccaattcaccatctccagagacaatgccaagaacaccctgtacctgcaaatgagccgtctgaagtctgaggacacagccatgtattactgtgcaagacgagaagattacgacggaagacttacttactggggccaagggactctggtcaccatctctgcaggaggaagtggtggaggcgggtcaggaggtggcgggagcggcggtgacattgtgctgacacagtctcctgcttccttagctgtatctctggggcagagggccaccatctcctgcagggccagcaaaagtgtcagtacatctggttatagttatatgaactggtaccaacagaaaccaggacagccacccaaagtcctcatctatcttgcatccaaactagaatctggggtccctgccaggttcagtggcagtgggtcagggacagacttcaccctcaacatccatcctgtggaggaggaggatgctgcaacctattactgtcagcacagtagggagcttccgtacacgttcggaggggggaccaaactggaaataaaaggtggtggcggttcagcacaccccggccgtcccagagcagtgcccacacagtgcgacgtcccccccaacagccgcttcgattgcgcccctgacaaggccatcacccaggaacagtgcgaggcccgcggctgttgctacatccctgcaaagcaggggctgcagggagcccagatggggcagccctggtgcttcttcccacccagctaccccagctacaagctggagaacctgagctcctctgaaatgggctacacggccaccctgacccgtaccacccccaccttcttccccaaggacatcctgaccctgcggctggacgtgatgatggagactgagaaccgcctccacttcacgatcaaagatccagctaacaggcgctacgaggtgcccttggagaccccgcatgtccacagccgggcaccgtccccactctacagcgtggagttctccgaggagcccttcggggtgatcgtgcgccggcagctggacggccgcgtgctgctgaacacgacggtggcgcccctgttctttgcggaccagttccttcagctgtccacctcgctgccctcgcagtatatcacaggcctcgccgagcacctcagtcccctgatgctcagcaccagctggaccaggatcaccctgtggaaccgggaccttgcgcccacgcccggtgcgaacctctacgggtctcaccctttctacctggcgctggaggacggcgggtcggcacacggggtgttcctgctaaacagcaatgccatggatgtggtcctgcagccgagccctgcccttagctggaggtcgacaggtgggatcctggatgtctacatcttcctgggcccagagcccaagagcgtggtgcagcagtacctggacgttgtgggatacccgttcatgccgccatactggggcctgggcttccacctgtgccgctggggctactcctccaccgctatcacccgccaggtggtggagaacatgaccagggcccacttccccctggacgtccagtggaacgacctggactacatggactcccggagggacttcacgttcaacaaggatggcttccgggacttcccggccatggtgcaggagctgcaccagggcggccggcgctacatgatgatcgtggatcctgccatcagcagctcgggccctgccgggagctacaggccctacgacgagggtctgcggaggggggttttcatcaccaacgagaccggccagccgctgattgggaaggtatggcccgggtccactgccttccccgacttcaccaaccccacagccctggcctggtgggaggacatggtggctgagttccatgaccaggtgcccttcgacggcatgtggattgacatgaacgagccttccaacttcatcaggggctctgaggacggctgccccaacaatgagctggagaacccaccctacgtgcctggggtggttggggggaccctccaggcggccaccatctgtgcctccagccaccagtttctctccacacactacaacctgcacaacctctacggcctgaccgaagccatcgcctcccacagggcgctggtgaaggctcgggggacacgcccatttgtgatctcccgctcgacctttgctggccacggccgatacgccggccactggacgggggacgtgtggagctcctgggagcagctcgcctcctccgtgccagaaatcctgcagtttaacctgctgggggtgcctctggtcggggccgacgtctgcggcttcctgggcaacacctcagaggagctgtgtgtgcgctggacccagctgggggccttctaccccttcatgcggaaccacaacagcctgctcagtctgccccaggagccgtacagcttcagcgagccggcccagcaggccatgaggaaggccctcaccctgcgctacgcactcctcccccacctctacacactgttccaccaggcccacgtcgcgggggagaccgtggcccggcccctcttcctggagttccccaaggactctagcacctggactgtggaccaccagctcctgtggggggaggccctgctcatcaccccagtgctccaggccgggaaggccgaagtgactggctacttccccttgggcacatggtacgacctgcagacggtgccagtagaggcccttggcagcctcccacccccacctgcagctccccgtgagccagccatccacagcgaggggcagtgggtgacgctgccggcccccctggacaccatcaacgtccacctccgggctgggtacatcatccccctgcagggccctggcctcacaaccacagagtcccgccagcagcccatggccctggctgtggccctgaccaagggtggggaggcccgaggggagctgttctgggacgatggagagagcctggaagtgctggagcgaggggcctacacacaggtcatcttcctggccaggaataacacgatcgtgaatgagctggtacgtgtgaccagtgagggagctggcctgcagctgcagaaggtgactgtcctgggcgtggccacggcgccccagcaggtcctctccaacggtgtccctgtctccaacttcacctacagccccgacaccaaggtcctggacatctgtgtctcgctgttgatgggagagcagtttctcgtcagctggtgttag

SEQ ID NO: 12 - DNA, 2859 bp, Homo sapiens
  source 1..2859: mol_type = other DNA
atgggagtgaggcacccgccctgctcccaccggctcctggccgtctgcgccctcgtgtccttggcaaccgctgcactcctggggcacatcctactccatgatttcctgctggttccccgagagctgagtggctcctccccagtcctggaggagactcacccagctcaccagcagggagccagcagaccagggccccgggatgcccaggcacaccccggccgtcccagagcagtgcccacacagtgcgacgtcccccccaacagccgcttcgattgcgcccctgacaaggccatcacccaggaacagtgcgaggcccgcggctgttgctacatccctgcaaagcaggggctgcagggagcccagatggggcagccctggtgcttcttcccacccagctaccccagctacaagctggagaacctgagctcctctgaaatgggctacacggccaccctgacccgtaccacccccaccttcttccccaaggacatcctgaccctgcggctggacgtgatgatggagactgagaaccgcctccacttcacgatcaaagatccagctaacaggcgctacgaggtgcccttggagaccccgcatgtccacagccgggcaccgtccccactctacagcgtggagttctccgaggagcccttcggggtgatcgtgcgccggcagctggacggccgcgtgctgctgaacacgacggtggcgcccctgttctttgcggaccagttccttcagctgtccacctcgctgccctcgcagtatatcacaggcctcgccgagcacctcagtcccctgatgctcagcaccagctggaccaggatcaccctgtggaaccgggaccttgcgcccacgcccggtgcgaacctctacgggtctcaccctttctacctggcgctggaggacggcgggtcggcacacggggtgttcctgctaaacagcaatgccatggatgtggtcctgcagccgagccctgcccttagctggaggtcgacaggtgggatcctggatgtctacatcttcctgggcccagagcccaagagcgtggtgcagcagtacctggacgttgtgggatacccgttcatgccgccatactggggcctgggcttccacctgtgccgctggggctactcctccaccgctatcacccgccaggtggtggagaacatgaccagggcccacttccccctggacgtccagtggaacgacctggactacatggactcccggagggacttcacgttcaacaaggatggcttccgggacttcccggccatggtgcaggagctgcaccagggcggccggcgctacatgatgatcgtggatcctgccatcagcagctcgggccctgccgggagctacaggccctacgacgagggtctgcggaggggggttttcatcaccaacgagaccggccagccgctgattgggaaggtatggcccgggtccactgccttccccgacttcaccaaccccacagccctggcctggtgggaggacatggtggctgagttccatgaccaggtgcccttcgacggcatgtggattgacatgaacgagccttccaacttcatcaggggctctgaggacggctgccccaacaatgagctggagaacccaccctacgtgcctggggtggttggggggaccctccaggcggccaccatctgtgcctccagccaccagtttctctccacacactacaacctgcacaacctctacggcctgaccgaagccatcgcctcccacagggcgctggtgaaggctcgggggacacgcccatttgtgatctcccgctcgacctttgctggccacggccgatacgccggccactggacgggggacgtgtggagctcctgggagcagctcgcctcctccgtgccagaaatcctgcagtttaacctgctgggggtgcctctggtcggggccgacgtctgcggcttcctgggcaacacctcagaggagctgtgtgtgcgctggacccagctgggggccttctaccccttcatgcggaaccacaacagcctgctcagtctgccccaggagccgtacagcttcagcgagccggcccagcaggccatgaggaaggccctcaccctgcgctacgcactcctcccccacctctacacactgttccaccaggcccacgtcgcgggggagaccgtggcccggcccctcttcctggagttccccaaggactctagcacctggactgtggaccaccagctcctgtggggggaggccctgctcatcaccccagtgctccaggccgggaaggccgaagtgactggctacttccccttgggcacatggtacgacctgcagacggtgccagtagaggcccttggcagcctcccacccccacctgcagctccccgtgagccagccatccacagcgaggggcagtgggtgacgctgccggcccccctggacaccatcaacgtccacctccgggctgggtacatcatccccctgcagggccctggcctcacaaccacagagtcccgccagcagcccatggccctggctgtggccctgaccaagggtggggaggcccgaggggagctgttctgggacgatggagagagcctggaagtgctggagcgaggggcctacacacaggtcatcttcctggccaggaataacacgatcgtgaatgagctggtacgtgtgaccagtgagggagctggcctgcagctgcagaaggtgactgtcctgggcgtggccacggcgccccagcaggtcctctccaacggtgtccctgtctccaacttcacctacagccccgacaccaaggtcctggacatctgtgtctcgctgttgatgggagagcagtttctcgtcagctggtgttag

SEQ ID NO: 13 - DNA, 354 bp, Homo sapiens
  source 1..354: mol_type = other DNA
caggtgcagctgcaggagtcgggccccggactgatgaagccttcggagaccctgtccctcacctgcactgtctctggtggctccttcagcagttactattggaactggatccggcagtccccagggaagggactggagtggattgggtatatccgttatagtggggacaccaactacaagccctccctcaagagtcgattcaccatatcaattgacacgtccaagaaccttttctccctgaggctgaaatctgtgaccgctgcggacacggccgtgtattactgtgcgaggatgggactggggagtgatgcttttgatatctggggccaagggacaatggtcaccgtctcttca

SEQ ID NO: 14 - protein, 118 aa, Homo sapiens
QVQLQESGPGLMKPSETLSLTCTVSGGSFSSYYWNWIRQSPGKGLEWIGYIRYSGDTNYKPSLKSRFTISIDTSKNLFSLRLKSVTAADTAVYYCARMGLGSDAFDIWGQGTMVTVSS

SEQ ID NO: 15 - DNA, 24 bp, Homo sapiens
  source 1..24: mol_type = other DNA
ggtggctccttcagcagttactat

SEQ ID NO: 16 - protein, 8 aa, Homo sapiens
GGSFSSYY

SEQ ID NO: 17 - DNA, 21 bp, Homo sapiens
  source 1..21: mol_type = other DNA
atccgttatagtggggacacc

SEQ ID NO: 18 - protein, 7 aa, Homo sapiens
IRYSGDT

SEQ ID NO: 19 - DNA, 36 bp, Homo sapiens
  source 1..36: mol_type = other DNA
gcgaggatgggactggggagtgatgcttttgatatc

SEQ ID NO: 20 - protein, 12 aa, Homo sapiens
ARMGLGSDAFDI

SEQ ID NO: 21 - DNA, 324 bp, Homo sapiens
  source 1..324: mol_type = other DNA
gaaattgtgttgacgcagtctccaggcaccctgtctttgtctccaggggaaagagccaccctctcctgcagggccagtcagagtgttaacaacaattatttagcctggtaccagcagaaacctggccaggctcccaggctcctcatctatggtgtattcaacagggccactaacatcccagacaggttcagtggcagtgggtctgggacagatttcactctcaccatcagcagactggagcctgaagattttgcagtgtattactgtcagcagtatggtagttcaccttggacgttcggccaagggaccaaggtggaaatcaaa

SEQ ID NO: 22 - protein, 108 aa, Homo sapiens
EIVLTQSPGTLSLSPGERATLSCRASQSVNNNYLAWYQQKPGQAPRLLIYGVFNRATNIPDRFSGSGSGTDFTLTISRLEPEDFAVYYCQQYGSSPWTFGQGTKVEIK

SEQ ID NO: 23 - DNA, 21 bp, Homo sapiens
  source 1..21: mol_type = other DNA
cagagtgttaacaacaattat

SEQ ID NO: 24 - protein, 7 aa, Homo sapiens
QSVNNNY

SEQ ID NO: 25-26 - skipped (2 entries)

SEQ ID NO: 27 - DNA, 27 bp, Homo sapiens
  source 1..27: mol_type = other DNA
cagcagtatggtagttcaccttggacg

SEQ ID NO: 28 - protein, 9 aa, Homo sapiens
QQYGSSPWT

SEQ ID NO: 29 - DNA, 354 bp, Homo sapiens
  source 1..354: mol_type = other DNA
caggtgcagctgcaggagtcgggcccaagactggtgaagccttcggagaccctgtccctcacctgcattgtctctggtggctccatcagtaatttctactggaactggatccggcagtccccagggaagggactggaatggattggatatttcttttacactgggactatcgactacaacccctccctcaagagtcgagtcaccatatcactggacacgtccaagaaccagttctccctgaacctgcgtcttctgaccgccgcagacgcggccgtttattattgtgcgaggatggggctgggggctaatgcttttgacatctggggccacgggacaatggtcaccgtctcttca

SEQ ID NO: 30 - protein, 118 aa, Homo sapiens
QVQLQESGPRLVKPSETLSLTCIVSGGSISNFYWNWIRQSPGKGLEWIGYFFYTGTIDYNPSLKSRVTISLDTSKNQFSLNLRLLTAADAAVYYCARMGLGANAFDIWGHGTMVTVSS

SEQ ID NO: 31 - DNA, 24 bp, Homo sapiens
  source 1..24: mol_type = other DNA
ggtggctccatcagtaatttctac

SEQ ID NO: 32 - protein, 8 aa, Homo sapiens
GGSISNFY

SEQ ID NO: 33 - DNA, 21 bp, Homo sapiens
  source 1..21: mol_type = other DNA
ttcttttacactgggactatc

SEQ ID NO: 34 - protein, 7 aa, Homo sapiens
FFYTGTI

SEQ ID NO: 35 - DNA, 36 bp, Homo sapiens
  source 1..36: mol_type = other DNA
gcgaggatggggctgggggctaatgcttttgacatc

SEQ ID NO: 36 - protein, 12 aa, Homo sapiens
ARMGLGANAFDI

SEQ ID NO: 37 - DNA, 324 bp, Homo sapiens
  source 1..324: mol_type = other DNA
gaaattgtgttgacgcagtctccaggcaccctgtctttgtctcctggagaaagagccaccctctcctgcagggccagtcagcatgttagcagcaactacttagcctggtaccagcagaaacctggccaggctcccaggctcctcatctatggtggatccagcagggccactggcatcccagacaggttcagtggcagtgggtctgggacagacttcactctcaccatcagcagactggagcctgcagattttgcagtgttttactgtcagcagtatggtaactcaccttggacgttcggccaagggaccaaggtggaaatgaaa

SEQ ID NO: 38 - protein, 108 aa, Homo sapiens
EIVLTQSPGTLSLSPGERATLSCRASQHVSSNYLAWYQQKPGQAPRLLIYGGSSRATGIPDRFSGSGSGTDFTLTISRLEPADFAVFYCQQYGNSPWTFGQGTKVEMK

SEQ ID NO: 39 - DNA, 21 bp, Homo sapiens
  source 1..21: mol_type = other DNA
cagcatgttagcagcaactac

SEQ ID NO: 40 - protein, 7 aa, Homo sapiens
QHVSSNY

SEQ ID NO: 41-42 - skipped (2 entries)

SEQ ID NO: 43 - DNA, 27 bp, Homo sapiens
  source 1..27: mol_type = other DNA
cagcagtatggtaactcaccttggacg

SEQ ID NO: 44 - protein, 9 aa, Homo sapiens
QQYGNSPWT

SEQ ID NO: 45 - DNA, 351 bp, Homo sapiens
  source 1..351: mol_type = other DNA
caggtgcaactacaggagtcgggcccaaaggtggtgaagccttcggagaccctgtccctcacctgcactgtctctggtggctccatcagtagttactactggaattggatccgccagtccccagggaagggactggagtggattggatataccaaaagagggtataccgactacaacccctccctcaggagtcgcgtcactatatcagaagacacgtccaagaaccagttctccctgaggatcagctctgtgaccgccgcagacacggccgtatattactgtgcacaaatggggtggggatcccatgcttttgacatgtggggccaagggacaatggtcgccgtctcttca

SEQ ID NO: 46 - protein, 117 aa, Homo sapiens
QVQLQESGPKVVKPSETLSLTCTVSGGSISSYYWNWIRQSPGKGLEWIGYTKRGYTDYNPSLRSRVTISEDTSKNQFSLRISSVTAADTAVYYCAQMGWGSHAFDMWGQGTMVAVSS

SEQ ID NO: 47 - DNA, 24 bp, Homo sapiens
  source 1..24: mol_type = other DNA
ggtggctccatcagtagttactac

SEQ ID NO: 48 - protein, 8 aa, Homo sapiens
GGSISSYY

SEQ ID NO: 49 - DNA, 18 bp, Homo sapiens
  source 1..18: mol_type = other DNA
accaaaagagggtatacc

SEQ ID NO: 50 - protein, 6 aa, Homo sapiens
TKRGYT

SEQ ID NO: 51 - DNA, 36 bp, Homo sapiens
  source 1..36: mol_type = other DNA
gcacaaatggggtggggatcccatgcttttgacatg

SEQ ID NO: 52 - protein, 12 aa, Homo sapiens
AQMGWGSHAFDM

SEQ ID NO: 53 - DNA, 324 bp, Homo sapiens
  source 1..324: mol_type = other DNA
gaaattgtgttgacgcagtctccaggcaccctgtctttgtctccaggggaaagagccaccctctcctgcagggccagtcagagtgttagcagcagctacttagcctggtaccagcagaaacctggccaggctcccaggctcctcatctatggtgcatccagcagggccactggcatcccagacaggttcagtggcagtgggtctgggacagacttcactctcaccatcagcagactggagcctgaagattttgcagtgtattactgtcagcagtatggtagctcaccttggacgttcggccaagggaccaaggtggaaatcaaa

SEQ ID NO: 54 - protein, 108 aa, Homo sapiens
EIVLTQSPGTLSLSPGERATLSCRASQSVSSSYLAWYQQKPGQAPRLLIYGASSRATGIPDRFSGSGSGTDFTLTISRLEPEDFAVYYCQQYGSSPWTFGQGTKVEIK

SEQ ID NO: 55 - DNA, 21 bp, Homo sapiens
  source 1..21: mol_type = other DNA
cagagtgttagcagcagctac

SEQ ID NO: 56 - protein, 7 aa, Homo sapiens
QSVSSSY

SEQ ID NO: 57-58 - skipped (2 entries)

SEQ ID NO: 59 - DNA, 27 bp, Homo sapiens
  source 1..27: mol_type = other DNA
cagcagtatggtagctcaccttggacg

SEQ ID NO: 60 - protein, 9 aa, Homo sapiens
QQYGSSPWT

SEQ ID NO: 61 - DNA, 351 bp, Homo sapiens; identical to SEQ ID NO: 45
  source 1..351: mol_type = other DNA

SEQ ID NO: 62 - protein, 117 aa, Homo sapiens; identical to SEQ ID NO: 46

SEQ ID NO: 63 - DNA, 24 bp, Homo sapiens
  source 1..24: mol_type = other DNA
ggtggctccatcagtagttactac

SEQ ID NO: 64 - protein, 8 aa, Homo sapiens
GGSISSYY

SEQ ID NO: 65 - DNA, 18 bp, Homo sapiens
  source 1..18: mol_type = other DNA
accaaaagagggtatacc

SEQ ID NO: 66 - protein, 6 aa, Homo sapiens
TKRGYT

SEQ ID NO: 67 - DNA, 36 bp, Homo sapiens; identical to SEQ ID NO: 51
  source 1..36: mol_type = other DNA

SEQ ID NO: 68 - protein, 12 aa, Homo sapiens
AQMGWGSHAFDM

SEQ ID NO: 69 - DNA, 324 bp, Homo sapiens
  source 1..324: mol_type = other DNA
gaaattgtgttgacgcagtctccaggcaccctgtctttgtctccaggggaaagagccaccctctcctgcagggccagtcagagtgttaatagtaggtacttagcctggtaccagcagaaacctggccaggctcccaggctcctcatctatggtgcatccagcagggccactggcatcccagacaggtgcagtggcagtgggtccgggacagacttcactctcaccatcagcagactggagcctgaagattttgcagtgtattactgtcagcagtatggtagctcaccttggacgttcggccaggggaccaaggtggaaatcaaa

SEQ ID NO: 70 - protein, 108 aa, Homo sapiens
EIVLTQSPGTLSLSPGERATLSCRASQSVNSRYLAWYQQKPGQAPRLLIYGASSRATGIPDRCSGSGSGTDFTLTISRLEPEDFAVYYCQQYGSSPWTFGQGTKVEIK

SEQ ID NO: 71 - DNA, 21 bp, Homo sapiens
  source 1..21: mol_type = other DNA
cagagtgttaatagtaggtac

SEQ ID NO: 72 - protein, 7 aa, Homo sapiens
QSVNSRY

SEQ ID NO: 73-74 - skipped (2 entries)

SEQ ID NO: 75 - DNA, 27 bp, Homo sapiens
  source 1..27: mol_type = other DNA
cagcagtatggtagctcaccttggacg

SEQ ID NO: 76 - protein, 9 aa, Homo sapiens
QQYGSSPWT

SEQ ID NO: 77 - protein, 238 aa, Homo sapiens
MAVEGGMKCVKFLLYVLLLAFCACAVGLIAVGVGAQLVLSQTIIQGATPGSLLPVVIIAVGVFLFLVAFVGCCGACKENYCLMITFAIFLSLIMLVEVAAAIAGYVFRDKVMSEFNNNFRQQMENYPKNNHTASILDRMQADFKCCGAANYTDWEKIPSMSKNRVPDSCCINVTVGCGINFNEKAIHKEGCVEKIGGWLRKNVLVVAAAALGIAFVEVLGIVFACCLVKSIRSGYEVM

SEQ ID NO: 78 - protein, 917 aa, Homo sapiens
LLVPRELSGSSPVLEETHPAHQQGASRPGPRDAQAHPGRPRAVPTQCDVPPNSRFDCAPDKAITQEQCEARGCCYIPAKQGLQGAQMGQPWCFFPPSYPSYKLENLSSSEMGYTATLTRTTPTFFPKDILTLRLDVMMETENRLHFTIKDPANRRYEVPLETPHVHSRAPSPLYSVEFSEEPFGVIVRRQLDGRVLLNTTVAPLFFADQFLQLSTSLPSQYITGLAEHLSPLMLSTSWTRITLWNRDLAPTPGANLYGSHPFYLALEDGGSAHGVFLLNSNAMDVVLQPSPALSWRSTGGILDVYIFLGPEPKSVVQQYLDVVGYPFMPPYWGLGFHLCRWGYSSTAITRQVVENMTRAHFPLDVQWNDLDYMDSRRDFTFNKDGFRDFPAMVQELHQGGRRYMMIVDPAISSSGPAGSYRPYDEGLRRGVFITNETGQPLIGKVWPGSTAFPDFTNPTALAWWEDMVAEFHDQVPFDGMWIDMNEPSNFIRGSEDGCPNNELENPPYVPGVVGGTLQAATICASSHQFLSTHYNLHNLYGLTEAIASHRALVKARGTRPFVISRSTFAGHGRYAGHWTGDVWSSWEQLASSVPEILQFNLLGVPLVGADVCGFLGNTSEELCVRWTQLGAFYPFMRNHNSLLSLPQEPYSFSEPAQQAMRKALTLRYALLPHLYTLFHQAHVAGETVARPLFLEFPKDSSTWTVDHQLLWGEALLITPVLQAGKAEVTGYFPLGTWYDLQTVPVEALGSLPPPPAAPREPAIHSEGQWVTLPAPLDTINVHLRAGYIIPLQGPGLTTTESRQQPMALAVALTKGGEARGELFWDDGESLEVLERGAYTQVIFLARNNTIVNELVRVTSEGAGLQLQKVTVLGVATAPQQVLSNGVPVSNFTYSPDTKVLDICVSLLMGEQFLVSWC

SEQ ID NO: 79 - protein, 1128 aa, synthetic construct
  REGION 1..1128: note = scFv_H4H123450(VH-linker-VL)_linker_GAA
QVQLQESGPKVVKPSETLSLTCTVSGGSISSYYWNWIRQSPGKGLEWIGYTKRGYTDYNPSLRSRVTISEDTSKNQFSLRISSVTAADTAVYYCAQMGWGSHAFDMWGQGTMVAVSSGGSGGGGSGGGGSGGEIVLTQSPGTLSLSPGERATLSCRASQSVSSSYLAWYQQKPGQAPRLLIYGASSRATGIPDRFSGSGSGTDFTLTISRLEPEDFAVYYCQQYGSSPWTFGQGTKVEIKGGGGSAHPGRPRAVPTQCDVPPNSRFDCAPDKAITQEQCEARGCCYIPAKQGLQGAQMGQPWCFFPPSYPSYKLENLSSSEMGYTATLTRTTPTFFPKDILTLRLDVMMETENRLHFTIKDPANRRYEVPLETPHVHSRAPSPLYSVEFSEEPFGVIVRRQLDGRVLLNTTVAPLFFADQFLQLSTSLPSQYITGLAEHLSPLMLSTSWTRITLWNRDLAPTPGANLYGSHPFYLALEDGGSAHGVFLLNSNAMDVVLQPSPALSWRSTGGILDVYIFLGPEPKSVVQQYLDVVGYPFMPPYWGLGFHLCRWGYSSTAITRQVVENMTRAHFPLDVQWNDLDYMDSRRDFTFNKDGFRDFPAMVQELHQGGRRYMMIVDPAISSSGPAGSYRPYDEGLRRGVFITNETGQPLIGKVWPGSTAFPDFTNPTALAWWEDMVAEFHDQVPFDGMWIDMNEPSNFIRGSEDGCPNNELENPPYVPGVVGGTLQAATICASSHQFLSTHYNLHNLYGLTEAIASHRALVKARGTRPFVISRSTFAGHGRYAGHWTGDVWSSWEQLASSVPEILQFNLLGVPLVGADVCGFLGNTSEELCVRWTQLGAFYPFMRNHNSLLSLPQEPYSFSEPAQQAMRKALTLRYALLPHLYTLFHQAHVAGETVARPLFLEFPKDSSTWTVDHQLLWGEALLITPVLQAGKAEVTGYFPLGTWYDLQTVPVEALGSLPPPPAAPREPAIHSEGQWVTLPAPLDTINVHLRAGYIIPLQGPGLTTTESRQQPMALAVALTKGGEARGELFWDDGESLEVLERGAYTQVIFLARNNTIVNELVRVTSEGAGLQLQKVTVLGVATAPQQVLSNGVPVSNFTYSPDTKVLDICVSLLMGEQFLVSWC

SEQ ID NO: 80 - protein, 125 aa, synthetic construct
  REGION 1..125: note = CD63 EC loop 2 MMH
RDKVMSEFNNNFRQQMENYPKNNHTASILDRMQADFKCCGAANYTDWEKIPSMSKNRVPDSCCINVTVGCGINFNEKAIHKEGCVEKIGGWLRKNVLEQKLISEEDLGGEQKLISEEDLHHHHHH

SEQ ID NO: 81 - protein, 324 aa, synthetic construct
  REGION 1..324: note = CD63 EC loop 2 hFC
RDKVMSEFNNNFRQQMENYPKNNHTASILDRMQADFKCCGAANYTDWEKIPSMSKNRVPDSCCINVTVGCGINFNEKAIHKEGCVEKIGGWLRKNVLDKTHTCPPCPAPELLGGPSVFLFPPKPKDTLMISRTPEVTCVVVDVSHEDPEVKFNWYVDGVEVHNAKTKPREEQYNSTYRVVSVLTVLHQDWLNGKEYKCKVSNKALPAPIEKTISKAKGQPREPQVYTLPPSRDELTKNQVSLTCLVKGFYPSDIAVEWESNGQPENNYKTTPPVLDSDGSFFLYSKLTVDKSRWQQGNVFSCSVMHEALHNHYTQKSLSLSPGK